European Patent Specification EP 3 875 152 B1, published April 10, 2024. Title: COMPOSITIONS AND METHODS FOR TARGETED CYTOKINE DELIVERY. Applicant: Washington University. Application 15870897.4. The sequence listing filed with the application follows.

SEQUENCE LISTING (34 sequences)

SEQ ID NO: 1 - DNA, 944 bp, Artificial Sequence
  SYNTHESIZED
cacaaactcgcattcaacttcaatctagaaataaatggcagtgatacacattctacagtagatgtatatcttgatgattctcaaattataacgtttgatggaaaagatatccgtccaaccatcccgttcatgataggtgatgaaattttcttaccgttttataaaaatgtgtttagtgagtttttctctctgtttagaagagttcctacaagtactccatatgaagacttgacatatttttatgaatgcgactatacagacaataaatctacatttgatcagttttatctttataatggcgaagaatatactgtcaaaacacaggaggccactaataaaaatatgtggctaactacttccgagtttagactaaaaaaatggttcgatggcgaagattgtataatgcatcttagatcgttagttagaaaaatggaggacagtaaacgaaacactggtggtaccggaagtagcggtagtagtgattacaaggacgatgacgacaagcaccaccatcatcatcatcaccacggtagcagcggcagcagtgcccccacctctagcagcacaaagaagacccagctgcaactggaacacctcctgctggacctgcagatgatcctgaacggcatcaacaactacaagaaccccaagctgaccgccatgctgaccaaaaagttttacatgcccaagaaggccaccgagcttaaacacctgcaatgccttgaggaggagctgaagccctggaggaggtactgaacctggcccagagcaagaactttcatctgaggcccagggacctgattagcaacatcaacgtgatcgtgttggagttgaagggcagcgagaccacgttcatgtgcgagtacgccgacgagacggccaccatagtggagtttcttaacaggtggatcaccttctcacagtctatcatcagcaccctgacc

SEQ ID NO: 2 - protein, 315 aa, Artificial Sequence
  SYNTHESIZED
HKLAFNFNLEINGSDTHSTVDVYLDDSQIITFDGKDIRPTIPFMIGDEIFLPFYKNVFSEFFSLFRRVPTSTPYEDLTYFYECDYTDNKSTFDQFYLYNGEEYTVKTQEATNKNMWLTTSEFRLKKWFDGEDCIMHLRSLVRKMEDSKRNTGGTGSSGSSDYKDDDDKHHHHHHHHGSSGSSAPTSSSTKKTQLQLEHLLLDLQMILNGINNYKNPKLTAMLTKKFYMPKKATELKHLQCLEEELKPLEEVLNLAQSKNFHLRPRDLISNINVIVLELKGSETTFMCEYADETATIVEFLNRWITFSQSIISTLT

SEQ ID NO: 3 - protein, 9 aa, Homo sapiens
SVYDFFVWL

SEQ ID NO: 4 - protein, 8 aa, Homo sapiens
SIINFEKL

SEQ ID NO: 5 - protein, 133 aa, Homo sapiens [sequence omitted]

SEQ ID NO: 6 - protein, 133 aa, Artificial Sequence
  SYNTHESIZED
APTSSSTKKTQLQLEHLLLDLQMILNGINNYKNPKLTAMLTKKFYMPKKATELKHLQCLEEELKPLEEVLNLAQSKNFHLRPRDLISNINVIVLELKGSETTFMCEYADETATIVEFLNRWITFSQSIISTLT

SEQ ID NO: 7 - protein, 151 aa, Artificial Sequence
  SYNTHESIZED
HKLAFNFNLEINGSDTHSTVDVYLDDSQIITFDGKDIRPTIPFMIGDEIFLPFYKNVFSEFFSLFRRVPTSTPYEDLTYFYECDYTDNKSTFDQFYLYNGEEYTVKTQEATNKNMWLTTSEFRLKKWFDGEDCIMHLRSLVRKMEDSKRNT

SEQ ID NO: 8 - protein, 28 aa, Artificial Sequence
  SYNTHESIZED
GSSGSSDYKDDDDKHHHHHHHHGSSGSS

SEQ ID NO: 9 - protein, 7 aa, Artificial Sequence
  SYNTHESIZED
DYKDDDK

SEQ ID NO: 10 - protein, 9 aa, Artificial Sequence
  SYNTHESIZED
YPYDVPDYA

SEQ ID NO: 11 - protein, 10 aa, Artificial Sequence
  SYNTHESIZED
EQKLISEEDL

SEQ ID NO: 12 - protein, 14 aa, Artificial Sequence
  SYNTHESIZED
GKPIPNPLLGLDST

SEQ ID NO: 13 - protein, 150 aa, Cowpox virus
GHKLAFNFNLEINGSDTHSTVDVYLDDSQIITFDGKDIRPTIPFMIGDEIFLPFYKNVFSEFFSLFRRVPTSTPYEDLTYFYECDYTDNKSTFDQFYLYNGEEYTVKTQEATNKNMWLTTSEFRLKKWFDGEDCIMHLRSLVRKMEDSKR

SEQ ID NO: 14 - protein, 150 aa, Monkeypox virus
HKLVHYFNLKINGSDITNTADILLDNYPIMTFDGKDIYPSIAFMVGNKLFLDLYKNIFVEFFRLFRVSVSSQYEELEYYYSCDYTNNRPTIKQHYFYNGEEYTEIDRSKKATNKNSWLITSGFRLQKWFDSEDCIIYLRSLVRRMEDSNK

SEQ ID NO: 15 - protein, 181 aa, Homo sapiens
MEPHSLRYNLTVLSWDGSVQSGFLTEVHLDGQPFLRCRDRQKCRAKPQGQWAEDVLGNKTWDRETRDLTGNGKDLRMTLAHIKDQKEGLHSLQEIRVCEIHEDNSTRSSQHFYYDGELFLSQNLETKEWTMPQSSRAQTLAMNVRNFLKEDAMKTKTHYHAMHADCLQELRRYLKSGVVLR

SEQ ID NO: 16 - protein, 180 aa, Homo sapiens
MEPHSLRYNLMVLSQDGSVQSGFLAEGHLDGQPFLRYDRQKRRAKPQGQWAEDVLGAETWDTETEDLTENGQDLRRTLTHIKDQKGGLHSLQEIRVCEIHEDSSTRGSRHFYYNGELFLSQNLETQESTVPQSSRAQTLAMNVTNFWKEDAMKTKTHYRAMQADCLQKLQRYLKSGVAIR

SEQ ID NO: 17 - protein, 178 aa, Homo sapiens
DAHSLWYNFTIIHLPRHGQQWCEVQSQVDQKNFLSYDCGSDKVLSMGHLEEQLYATDAWGKQLEMLREVGQRLRLELADTELEDFTPSGPLTLQVRMSCECEADGYIRGSWQFSFDGRKFLLFDSNNRKWTVVHAGARRMKEKWEKDSGLTTFFKMVSMRDCKSWLRDFLMHRKKRLE

SEQ ID NO: 18 - protein, 174 aa, Homo sapiens
DAHSLRCNLTIKDPTPADPLWYEAKCFVGEILILHLSNINKTMTSGDPGETANATEVKKCLTQPLKNLCQKLRNKVSNTKVDTHKTNGYPHLQVTMIYPQSQGRTPSATWEFNISDSYFFTFYTENMSWRSANDESGVIMNKWKDDGEFVKQLKFLIHECSQKMDEFLKQSKEK

SEQ ID NO: 19 - protein, 16 aa, Homo sapiens
LTIIEMQKGDCALYAS

SEQ ID NO: 20 - protein, 16 aa, Chlorocebus sabaeus
LTIIEMQKGECALYAS

SEQ ID NO: 21 - protein, 16 aa, Callithrix jacchus
LTIIEMQKGDCAVYAS

SEQ ID NO: 22 - protein, 16 aa, Mus musculus
LTLVEIPKGSCAVYGS

SEQ ID NO: 23 - protein, 16 aa, Rattus norvegicus
LTLVKTPSGTCAVYGS

SEQ ID NO: 24 - protein, 16 aa, Cavia porcellus
LTLMDTQNGKCALYGS

SEQ ID NO: 25 - protein, 16 aa, Spermophilus sensu stricto
LTLVEMQNGTCIVYGS

SEQ ID NO: 26 - protein, 16 aa, Peromyscus maniculatus
LTVVEMQSGSCAVYGS

SEQ ID NO: 27 - protein, 16 aa, Heterocephalus glaber
LSMVEMQNGTCAVYAS

SEQ ID NO: 28 - protein, 16 aa, Microtus ochrogaster
LTLVEMQRGSCAVYGS

SEQ ID NO: 29 - protein, 16 aa, Sorex araneus
VSIVEMQGGNCAVYGS

SEQ ID NO: 30 - protein, 16 aa, Condylura cristata
VTVYEMQNGSCAVYGS

SEQ ID NO: 31 - protein, 16 aa, Cricetulus griseus
LTLVEMQNGSCAVYGS

SEQ ID NO: 32 - protein, 16 aa, Felis catus
LTMVDMQNGTCAVYGS

SEQ ID NO: 33 - protein, 5 aa, Cowpox virus
ASSFK

SEQ ID NO: 34 - protein, 4 aa, Artificial Sequence
  SYNTHESIZED
YINM